European Patent Specification EP 2 747 775 B1, published March 22, 2023. Title: Means and Methods for Treating Angiogenesis-Related Diseases. Applicant: Deutsches Krebsforschungszentrum. The sequence listing filed with the application follows.

SEQUENCE LISTING (17 sequences)

SEQ ID NO: 1 - protein, 1527 aa, mouse
MAPDPSRRLCLLLLLLLSCRLVPASADGNSLSPLNPLVWLWPPKTSDSLEGPVSKPQNSSPVQSTENPTTHVVPQDGLTEQQTTPASSELPPEEEEEEDQKAGQGGSPATPAVPIPLVAPAASPDMKEENVAGVGAKILNVAQGIRSFVQLWDEDSTIGHSAGTEVPDSSIPTVLPSPAELSSAPQGSKTTLWLSSAIPSSPDAQTTEAGTLAVPTQLPPFQSNLQAPLGRPSAPPDFPENVAEEVGLLQLLGDPLPEKISQIDDPHVGPAYIFGPDSNSGQVAQYHFPKLFFRDFSLLFHVRPATEAAGVLFAITDAAQVVVSLGVKLSEVRDGQQNISLLYTEPGASQTQTGASFRLPAFVGQWTHFALSVDGGSVALYVDCEEFQRVPFARASQGLELERGAGLFVGQAGTADPDKFQGMISELKVRKTPRVSPVHCLDEEDDDEDRASGDFGSGFEESSKSHKEDTSLLPGLPQPPPVTSPPLAGGSTTEDPRTEETEEDAAVDSIGAETLPGTGSSGAWDEAIQNPGRGLIKGGMKGQKGEPGAQGPPGPAGPQGPAGPVVQSPNSQPVPGAQGPPGPQGPPGKDGTPGRDGEPGDPGEDGRPGDTGPQGFPGTPGDVGPKGEKGDPGIGPRGPPGPPGPPGPSFRQDKLTFIDMEGSGFSGDIESLRGPRGFPGPPGPPGVPGLPGEPGRFGINGSYAPGPAGLPGVPGKEGPPGFPGPPGPPGPPGKEGPPGVAGQKGSVGDVGIPGPKGSKGDLGPIGMPGKSGLAGSPGPVGPPGPPGPPGPPGPGFAAGFDDMEGSGIPLWTTARSSDGLQGPPGSPGLKGDPGVAGLPGAKGEVGADGAQGIPGPPGREGAAGSPGPKGEKGMPGEKGNPGKDGVGRPGLPGPPGPPGPVIYVSSEDKAIVSTPGPEGKPGYAGFPGPAGPKGDLGSKGEQGLPGPKGEKGEPGTIFSPDGRALGHPQKGAKGEPGFRGPPGPYGRPGHKGEIGFPGRPGRPGTNGLKGEKGEPGDASLGFSMRGLPGPPGPPGPPGPPGMPIYDSNAFVESGRPGLPGQQGVQGPSGPKGDKGEVGPPGPPGQFPIDLFHLEAEMKGDKGDRGDAGQKGERGEPGAPGGGFFSSSVPGPPGPPGYPGIPGPKGESIRGPPGPPGPQGPPGIGYEGRQGPPGPPGPPGPPSFPGPHRQTVSVPGPPGPPGPPGPPGAMGASAGQVRIWATYQTMLDKIREVPEGWLIFVAEREELYVRVRNGFRKVLLEARTALPRGTGNEVAALQPPLVQLHEGSPYTRREYSYSTARPWRADDILANPPRLPDRQPYPGVPHHHSSYVHLPPARPTLSLAHTHQDFQPVLHLVALNTPLSGGMRGIRGADFQCFQQARAVGLSGTFRAFLSSRLQDLYSIVRRADRGSVPIVNLKDEVLSPSWDSLFSGSQGQLQPGARIFSFDGRDVLRHPAWPQKSVWHGSDPSGRRLMESYCETWRTETTGATGQASSLLSGRLLEQKAASCHNSYIVLCIENSFMTSFSK

SEQ ID NO: 2 - protein, 1516 aa, human
MAPYPCGCHILLLLFCCLAAARANLLNLNWLWFNNEDTSHAATTIPEPQGPLPVQPTADTTTHVTPRNGSTEPATAPGSPEPPSELLEDGQDTPTSAESPDAPEENIAGVGAEILNVAKGIRSFVQLWNDTVPTESLARAETLVLETPVGPLALAGPSSTPQENGTTLWPSRGIPSSPGAHTTEAGTLPAPTPSPPSLGRPWAPLTGPSVPPPSSERISEEVGLLQLLGDPPPQQVTQTDDPDVGLAYVFGPDANSGQVARYHFPSLFFRDFSLLFHIRPATEGPGVLFAITDSAQAMVLLGVKLSGVQDGHQDISLLYTEPGAGQTHTAASFRLPAFVGQWTHLALSVAGGFVALYVDCEEFQRMPLARSSRGLELEPGAGLFVAQAGGADPDKFQGVIAELKVRRDPQVSPMHCLDEEGDDSDGASGDSGSGLGDARELLREETGAALKPRLPAPPPVTTPPLAGGSSTEDSRSEEVEEQTTVASLGAQTLPGSDSVSTWDGSVRTPGGRVKEGGLKGQKGEPGVPGPPGRAGPPGSPCLPGPPGLPCPVSPLGPAGPALQTVPGPQGPPGPPGRDGTPGRDGEPGDPGEDGKPGDTGPQGFPGTPGDVGPKGDKGDPGVGERGPPGPQGPPGPPGPSFRHDKLTFIDMEGSGFGGDLEALRGPRGFPGPPGPPGVPGLPGEPGRFGVNSSDVPGPAGLPGVPGREGPPGFPGLPGPPGPPGREGPPGRTGQKGSLGEAGAPGHKGSKGAPGPAGARGESGLAGAPGPAGPPGPPGPPGPPGPGLPAGFDDMEGSGGPFWSTARSADGPQGPPGLPGLKGDPGVPGLPGAKGEVGADGVPGFPGLPGREGIAGPQGPKGDRGSRGEKGDPGKDGVGQPGLPGPPGPPGPVVYVSEQDGSVLSVPGPEGRPGFAGFPGPAGPKGNLGSKGERGSPGPKGEKGEPGSIFSPDGGALGPAQKGAKGEPGFRGPPGPYGRPGYKGEIGFPGRPGRPGMNGLKGEKGEPGDASLGFGMRGMPGPPGPPGPPGPPGTPVYDSNVFAESSRPGPPGLPGNQGPPGPKGAKGEVGPPGPPGQFPFDFLQLEAEMKGEKGDRGDAGQKGERGEPGGGGFFGSSLPGPPGPPGPRGYPGIPGPKGESIRGQPGPPGPQGPPGIGYEGRQGPPGPPGPPGPPSFPGPHRQTISVPGPPGPPGPPGPPGTMGASSGVRLWATRQAMLGQVHEVPEGWLIFVAEQEELYVRVQNGFRKVQLEARTPLPRGTDNEVAALQPPVVQLHDSNPYPRREHPHPTARPWRADDILASPPRLPEPQPYPGAPHHSSYVHLRPARPTSPPAHSHRDFQPVLHLVALNSPLSGGMRGIRGADFQCFQQARAVGLAGTFRAFLSSRLQDLYSIVRRADRAAVPIVNLKDELLFPSWEALFSGSEGPLKPGARIFSFDGKDVLRHPTWPQKSVWHGSDPNGRRLTESYCETWRTEAPSATGQASSLLGGRLLGQSAASCHHAYIVLCIENSFMTASK

SEQ ID NO: 3 - protein, 315 aa, mouse
AGQVRIWATYQTMLDKIREVPEGWLIFVAEREELYVRVRNGFRKVLLEARTALPRGTGNEVAALQPPLVQLHEGSPYTRREYSYSTARPWRADDILANPPRLPDRQPYPGVPHHHSSYVHLPPARPTLSLAHTHQDFQPVLHLVALNTPLSGGMRGIRGADFQCFQQARAVGLSGTFRAFLSSRLQDLYSIVRRADRGSVPIVNLKDEVLSPSWDSLFSGSQGQLQPGARIFSFDGRDVLRHPAWPQKSVWHGSDPSGRRLMESYCETWRTETTGATGQASSLLSGRLLEQKAASCHNSYIVLCIENSFMTSFSK

SEQ ID NO: 4 - protein, 312 aa, human
SGVRLWATRQAMLGQVHEVPEGWLIFVAEQEELYVRVQNGFRKVQLEARTPLPRGTDNEVAALQPPVVQLHDSNPYPRREHPHPTARPWRADDILASPPRLPEPQPYPGAPHHSSYVHLRPARPTSPPAHSHRDFQPVLHLVALNSPLSGGMRGIRGADFQCFQQARAVGLAGTFRAFLSSRLQDLYSIVRRADRAAVPIVNLKDELLFPSWEALFSGSEGPLKPGARIFSFDGKDVLRHPTWPQKSVWHGSDPNGRRLTESYCETWRTEAPSATGQASSLLGGRLLGQSAASCHHAYIVLCIENSFMTASK

SEQ ID NO: 5 - protein, 233 aa, mouse
EPRGPTIKPCPPCKCPAPNLLGGPSVFIFPPKIKDVLMISLSPIVTCVVVDVSEDDPDVQISWFVNNVEVHTAQTQTHREDYNSTLRVVSALPIQHQDWMSGKEFKCKVNNKDLPAPIERTISKPKGSVRAPQVYVLPPPEEEMTKKQVTLTCMVTDFMPEDIYVEWTNNGKTELNYKNTEPVLDSDGSYFMYSKLRVEKKNWVERNSYSCSVVHEGLHNHHTTKSFSRTPGK

SEQ ID NO: 6 - protein, 232 aa, human
EPKSSDKTHTCPPCPAPELLGGPSVFLFPPKPKDTLMISRTPEVTCVVVDVSHEDPEVKFNWYVDGVEVHNAKTKPREEQYNSTYRVVSVLTVLHQDWLNGKEYKCKVSNKALPAPIEKTISKAKGQPREPQVYTLPPSREEMTKNQVSLTCLVKGFYPSDIAVEWESNGQPENNYKTTPPVLDSDGSFFLYSKLTVDKSRWQQGNVFSCSVMHEALHNHYTQKSLSLSPGK

SEQ ID NO: 7 - protein, 28 aa, mouse
HTHQDFQPVLHLVLYAVTGRGDSPASSK

SEQ ID NO: 8 - protein, 15 aa, mouse
LYAVTGRGDSPASSK

SEQ ID NO: 9 - protein, 26 aa, mouse
HTHQDFQPVLHLVALNTPLSGGMRGI

SEQ ID NO: 10 - protein, 25 aa, human
HSHRDFQPVLHLVALNSPLSGGMRG

SEQ ID NO: 11 - protein, 15 aa, mouse
LYAVTGRGDSPASSK

SEQ ID NO: 12 - protein, 15 aa, human
VYAVTGRGDSPASSK

SEQ ID NO: 13 - protein, 27 aa, human
HSHRDFQPVLHLVYAVTGRGDSPASSK

SEQ ID NO: 14 - protein, 27 aa, human
ASARDFQPVLHLVYAVTGRGDSPASSK

SEQ ID NO: 15 - protein, 27 aa, human
HSHRDFCPVLHLVYAVTGRGDSPASSK

SEQ ID NO: 16 - protein, 27 aa, human
HSHRDFQPVLHLVYAVTGRADSPASSK

SEQ ID NO: 17 - protein, 25 aa, mouse
IKPGADYTITLYAVTGRGDSPASSK